European Patent Specification EP 3 837 970 B1, published July 19, 2023. Title: Herbicide Tolerance Genes and Methods of Use Thereof. Applicant: Monsanto Technology LLC. The sequence listing filed with the application follows.

SEQUENCE LISTING (61 sequences)

SEQ ID NO: 1 - protein, 295 aa, Artificial Sequence
  Recombinant
MHAALSPLSQRFERIAVQPLTGVLGAEITGVDLREPLSDSTWNEILDAFHTYQVIYFPGQAITNEQHIAFSRRFGPVDPVPLLKSIEGYPEVQMIRREANESGRVIGDDWHTDSSFLDAPPAAVVMRAIDVPEHGGDTGFLSMYTAYDALSDGLKKLISGLNVVHSATRVFGSLYQAQNRRFSNTSVKVMDVADGDRETVHPLVVTHPGSGRKGLYVNQVYCQRIEGMSEKESEPLLSFLFAHATKPEFTCRVRWKKDQVLVWDNLCTMHYAINDYHGQTRILHRTTVGGVRPAR

SEQ ID NO: 2 - DNA, 906 bp, Artificial Sequence
  Recombinant
atgcatgctgcactgtcccccctctcccagcgctttgagcgcatcgcggtccagccgctgaccggcgtcctgggcgccgagatcaccggcgtcgacctgcgcgagccgctcagcgacagcacctggaacgaaatcctcgacgcgttccacacttaccaggtcatctattttcccggccaggcgatcaccaacgaacagcacatcgccttcagccggcgcttcggccccgtcgatcccgtgcccctgctcaagagcatcgaagggtatccagaggtgcagatgatccgccgcgaagccaacgaaagcgggcgtgtgatcggtgatgactggcacaccgacagcagcttcctggacgcaccgccggccgccgtggtgatgcgcgcgatcgacgtgcccgagcatggcggcgacaccggttttctgagcatgtacaccgcgtatgatgcgctgtcggatggcctgaagaaactgatcagcgggttgaacgtagtgcacagcgccacgcgtgtgttcggctcgctctaccaggcccagaaccggcgcttcagcaacaccagcgtcaaggtgatggacgtcgcagatggcgaccgtgaaaccgtgcaccccctggtggtgacccatccgggcagcggccgcaagggcctgtacgtgaaccaggtctattgccagcgcatcgagggcatgagcgaaaaagaaagcgaaccgctgctgagcttcctgtttgcgcatgcgacaaaaccggaattcacctgccgcgtgcgctggaagaaggaccaggtcctggtctgggacaacctgtgcacgatgcactatgccattaacgactaccatggccagacccgcattctgcatcgcaccacggtcggtggcgtgcgcccggcgcgccatcatcaccatcatcactag

SEQ ID NO: 3 - DNA, 888 bp, Artificial Sequence
  Recombinant
atgcacgccgctctgagcccgcttagccagcgcttcgagcgcatcgccgtgcagccgctgaccggcgtgctaggcgctgagatcaccggcgttgacctgagggagccgcttagcgactccacctggaacgagatcctcgacgccttccacacttaccaagttatctacttcccaggacaggctatcacgaacgaacagcacatcgccttctcgcggaggttcgggccagtggacccagtcccgctgcttaagtctatcgaaggctaccctgaggtgcaaatgatccgccgcgaggcgaacgaatccgggagggttattggcgacgattggcacactgactccagcttcctcgatgctcctccagcagccgtcgtgatgcgggccatcgacgtgccggagcacggcggcgatacgggtttcctgtccatgtacactgcttacgacgctctttctgatggcctcaagaaactcatcagcggactcaatgtggtccactctgcgacccgtgtctttggctcgctctatcaggcgcagaataggcgcttcagcaacacctccgtgaaggtcatggacgtggcggatggagacagggagactgtccacccgctcgtcgttactcaccctgggtccggccgtaagggtctgtacgtgaaccaggtgtactgtcagcgaattgagggtatgagtgagaaggagtccgagccgctgctcagtttcctcttcgcgcacgccaccaagcccgagttcacctgccgcgtccgctggaagaaggatcaagtcctggtgtgggacaacctctgcaccatgcactacgccatcaatgactatcatggtcaaacccggattcttcatcgcacaacggttggcggcgtgagacctgcccggtga

SEQ ID NO: 4 - protein, 295 aa, Artificial Sequence
  Recombinant
MHAALSPLSQRFERIAVQPLTGVLGAEITGVDLREPLDDSTWNEILDAFHTYQVIYFPGQAITNEQQIAFSRRFGPVDPVPLLKSIEGYPEVQMIRREANESGRVIGDDWHTDSTFLDAPPAAVVMRAIDVPEHGGDTGFLSMYTAYDALSDGLKKLISGLNVVHSATRVFGSLYQAQNRRFSNTSVKVMDVDAGDRETVHPLVVTHPGSGRKGLYVNQVYCQRIEGMSEKESEPLLSFLFAHATKPEFTCRVRWKKDQVLVWDNLCTMHYAINDYHGQTRILHRTTVGGVRPAR

SEQ ID NO: 5 - DNA, 906 bp, Artificial Sequence
  Recombinant
atgcatgctgcactgtcccccctctcccagcgctttgagcgcatcgcggtccagccgctgaccggcgtcctgggcgccgagatcaccggcgtcgacctgcgcgagccgctcgacgacagcacctggaacgaaatcctcgacgcgttccacacttaccaggtcatctattttcccggccaggcgatcaccaacgaacagcagatcgccttcagccggcgcttcggccccgtcgatcccgtgcccctgctcaagagcatcgaagggtatccagaggtgcagatgatccgccgcgaagccaacgaaagcgggcgtgtgatcggtgatgactggcacaccgacagcaccttcctggacgcaccgccggccgccgtggtgatgcgcgcgatcgacgtgcccgagcatggcggcgacaccggttttctgagcatgtacaccgcgtatgatgcgctgtcggatggcctgaagaaactgatcagcgggttgaacgtagtgcacagcgccacgcgtgtgttcggctcgctctaccaggcccagaaccggcgcttcagcaacaccagcgtcaaggtgatggacgtcgacgcgggcgaccgtgaaaccgtgcaccccctggtggtgacccatccgggcagcggccgcaagggcctgtacgtgaaccaggtctattgccagcgcatcgagggcatgagcgaaaaagaaagcgaaccgctgctgagcttcctgtttgcgcatgcgacaaaaccggaattcacctgccgcgtgcgctggaagaaggaccaggtcctggtctgggacaacctgtgcacgatgcactatgccattaacgactaccatggccagacccgcattctgcatcgcaccacggtcggtggcgtgcgcccggcgcgccatcatcaccatcatcactag

SEQ ID NO: 6 - DNA, 888 bp, Artificial Sequence
  Recombinant
atgcacgccgctctgagcccgcttagccagcgcttcgagcgcatcgccgtgcagccgctgaccggcgtgctaggcgctgagatcaccggcgttgacctgagggagccgcttgacgactccacctggaacgagatcctcgacgccttccacacttaccaagttatctacttcccaggacaggctatcacgaacgaacagcagatcgccttctcgcggaggttcgggccagtggacccagtcccgctgcttaagtctatcgaaggctaccctgaggtgcaaatgatccgccgcgaggcgaacgaatccgggagggttattggcgacgattggcacactgactccaccttcctcgatgctcctccagcagccgtcgtgatgcgggccatcgacgtgccggagcacggcggcgatacgggtttcctgtccatgtacactgcttacgacgctctttctgatggcctcaagaaactcatcagcggactcaatgtggtccactctgcgacccgtgtctttggctcgctctatcaggcgcagaataggcgcttcagcaacacctccgtgaaggtcatggacgtggacgcgggagacagggagactgtccacccgctcgtcgttactcaccctgggtccggccgtaagggtctgtacgtgaaccaggtgtactgtcagcgaattgagggtatgagtgagaaggagtccgagccgctgctcagtttcctcttcgcgcacgccaccaagcccgagttcacctgccgcgtccgctggaagaaggatcaagtcctggtgtgggacaacctctgcaccatgcactacgccatcaatgactatcatggtcaaacccggattcttcatcgcacaacggttggcggcgtgagacctgcccggtga

SEQ ID NO: 7 - protein, 295 aa, Artificial Sequence
  Recombinant
MHAALSPLSQRFERIAVQPLTGVLGAEITGVDLREPLSDSTWNEILDAFHTYQVIYFPGQAITNEQHIAFSRRFGPVDPVPLLKSIEGYPEVQMIRREANESGRVIGDDWHSDSTFLDAPPAAVVMRAIDVPEHGGDTGFLSMYTAYDALSDGLKKLISGLNVVHSATRVFGSLYQAQNRRFSNTSVKVMDVDAGDRETVHPLVVTHPGSGRKGLYVNQVYCQRIEGMSEKESEPLLSFLFAHATKPEFTCRVRWKKDQVLVWDNLCTMHYAINDYHGQTRILHRTTVGGVRPAR

SEQ ID NO: 8 - DNA, 906 bp, Artificial Sequence
  Recombinant
atgcatgctgcactgtcccccctctcccagcgctttgagcgcatcgcggtccagccgctgaccggcgtcctgggcgccgagatcaccggcgtcgacctgcgcgagccgctcagcgacagcacctggaacgaaatcctcgacgcgttccacacttaccaggtcatctattttcccggccaggcgatcaccaacgaacagcacatcgccttcagccggcgcttcggccccgtcgatcccgtgcccctgctcaagagcatcgaagggtatccagaggtgcagatgatccgccgcgaagccaacgaaagcgggcgtgtgatcggtgatgactggcacagcgacagcaccttcctggacgcaccgccggccgccgtggtgatgcgcgcgatcgacgtgcccgagcatggcggcgacaccggttttctgagcatgtacaccgcgtatgatgcgctgtcggatggcctgaagaaactgatcagcgggttgaacgtagtgcacagcgccacgcgtgtgttcggctcgctctaccaggcccagaaccggcgcttcagcaacaccagcgtcaaggtgatggacgtcgacgcgggcgaccgtgaaaccgtgcaccccctggtggtgacccatccgggcagcggccgcaagggcctgtacgtgaaccaggtctattgccagcgcatcgagggcatgagcgaaaaagaaagcgaaccgctgctgagcttcctgtttgcgcatgcgacaaaaccggaattcacctgccgcgtgcgctggaagaaggaccaggtcctggtctgggacaacctgtgcacgatgcactatgccattaacgactaccatggccagacccgcattctgcatcgcaccacggtcggtggcgtgcgcccggcgcgccatcatcaccatcatcactag

SEQ ID NO: 9 - protein, 295 aa, Artificial Sequence
  Recombinant
MHAALSPLSQRFERIAVQPLTGVLGAEITGVDLREPLDDSTWNEILDAFHTYQVIYFPGQAITNEQHIAFSRRFGPVDPVPLLKSIEGYPEVQMIRREANESGRVLGDDWHTDSTFLDAPPAAVVMRAIDVPEHGGDTGFLSMYTAYDALSDGLKKLISGLNVVHSATRVFGSLYQAQNRRFSNTSVKVMDVADGDRETVHPLVVTHPGSGRKGLYVNQVYCQRIEGMSEKESEPLLSFLFAHATKPEFTCRVRWKKDQVVVWDNLCTMHYAINDYHGQTRILHRTTVGGVRPAR

SEQ ID NO: 10 - DNA, 906 bp, Artificial Sequence
  Recombinant
atgcatgctgcactgtcccccctctcccagcgctttgagcgcatcgcggtccagccgctgaccggcgtcctgggcgccgagatcaccggcgtcgacctgcgcgagccgctcgacgacagcacctggaacgaaatcctcgacgcgttccacacttaccaggtcatctattttcccggccaggcgatcaccaacgaacagcacatcgccttcagccggcgcttcggccccgtcgatcccgtgcccctgctcaagagcatcgaagggtatccagaggtgcagatgatccgccgcgaagccaacgaaagcgggcgtgtgctgggtgatgactggcacaccgacagcaccttcctggacgcaccgccggccgccgtggtgatgcgcgcgatcgacgtgcccgagcatggcggcgacaccggttttctgagcatgtacaccgcgtatgatgcgctgtcggatggcctgaagaaactgatcagcgggttgaacgtagtgcacagcgccacgcgtgtgttcggctcgctctaccaggcccagaaccggcgcttcagcaacaccagcgtcaaggtgatggacgtcgcagatggcgaccgtgaaaccgtgcaccccctggtggtgacccatccgggcagcggccgcaagggcctgtacgtgaaccaggtctattgccagcgcatcgagggcatgagcgaaaaagaaagcgaaccgctgctgagcttcctgtttgcgcatgcgacaaaaccggaattcacctgccgcgtgcgctggaagaaggaccaggtcgtggtctgggacaacctgtgcacgatgcactatgccattaacgactaccatggccagacccgcattctgcatcgcaccacggtcggtggcgtgcgcccggcgcgccatcatcaccatcatcactag

SEQ ID NO: 11 - protein, 295 aa, Artificial Sequence
  Recombinant
MHAALSPLSQRFERIAVQPLTGVLGAEITGVDLREPLDDSTWNEILDAFHTYQVIYFPGQAITNEQHIAFSRRFGPVDPVPLLKSIEGYPEVQMIRREANESGRVIGENWHTDSTFLDAPPAAVVMYAKEIPPYGGDTLFTSMYTAWETLSPTMQATIEGLNVVHSATRVFGSLYQAQNRRFSNTSVKVMDVDAGDRETVHPLVVTHPETGRKGLYVNQVYCQRIEGMSEKESEPLLSFLFAHATKPEFTCRVRWQEGDVLVWDNLCTQHYAVPDYAGKFRYLTRTTVGGVRPAR

SEQ ID NO: 12 - DNA, 906 bp, Artificial Sequence
  Recombinant
atgcatgctgcactgtcccccctctcccagcgctttgagcgcatcgcggtccagccgctgaccggcgtcctgggcgccgagatcaccggcgtcgacctgcgcgagccgctcgacgacagcacctggaacgaaatcctcgacgcgttccacacttaccaggtcatctattttcccggccaggcgatcaccaacgaacagcacatcgccttcagccggcgcttcggccccgtcgatcccgtgcccctgctcaagagcatcgaagggtatccagaggtgcagatgatccgccgcgaagccaacgaaagcgggcgtgtgatcggtgaaaactggcacaccgacagcaccttcctggacgcaccgccggccgccgtggtgatgtatgcgaaagaaattcccccgtatggcggcgacaccctgtttaccagcatgtacaccgcgtgggagacgctgtcgcccaccatgcaggccaccatcgaagggttgaacgtagtgcacagcgccacgcgtgtgttcggctcgctctaccaggcccagaaccggcgcttcagcaacaccagcgtcaaggtgatggacgtcgacgcgggcgaccgtgaaaccgtgcaccccctggtggtgacccatccggaaaccggccgcaagggcctgtacgtgaaccaggtctattgccagcgcatcgagggcatgagcgaaaaagaaagcgaaccgctgctgagcttcctgtttgcgcatgcgacaaaaccggaattcacctgccgcgtgcgctggcaggaaggcgatgtcctggtctgggacaacctgtgcacgcagcactatgccgtacccgactacgcgggcaagttccgctacctgacgcgcaccacggtcggtggcgtgcgcccggcgcgccatcatcaccatcatcactag

SEQ ID NO: 13 - DNA, 888 bp, Artificial Sequence
  Recombinant
atgcacgccgctctgagcccgcttagccagcgcttcgagcgcatcgccgtgcagccgctgaccggcgtgctaggcgctgagatcaccggcgttgacctgagggagccgcttgacgactccacctggaacgagatcctcgacgccttccacacttaccaagttatctacttcccaggacaggctatcacgaacgaacagcacatcgccttctcgcggaggttcgggccagtggacccagtcccgctgcttaagtctatcgaaggctaccctgaggtgcaaatgatccgccgcgaggcgaacgaatccgggagggttattggcgagaactggcacactgactccaccttcctcgatgctcctccagcagccgtcgtgatgtacgccaaggagatcccgccctacggcggcgatacgctcttcacctccatgtacactgcttgggagaccctttctccgaccatgcaagccaccatcgagggactcaatgtggtccactctgcgacccgtgtctttggctcgctctatcaggcgcagaataggcgcttcagcaacacctccgtgaaggtcatggacgtggacgccggagacagggagactgtccacccgctcgtcgttactcaccctgagaccggccgtaagggtctgtacgtgaaccaggtgtactgtcagcgaattgagggtatgagtgagaaggagtccgagccgctgctcagtttcctcttcgcgcacgccaccaagcccgagttcacctgccgcgtccgctggcaagagggcgacgtcctggtgtgggacaacctctgcacccagcactacgccgtgccggactatgccgggaagttccgctaccttacccgcacaacggttggcggcgtgagacctgcccggtga

SEQ ID NO: 14 - protein, 295 aa, Artificial Sequence
  Recombinant
MHAALTPLTNKYRFIDVQPLTGVLGAEITGVDLREPLDDSTWNEILDAFHTYQVIYFPGQAITNEQHIAFSRRFGPVDPVPILKSIEGYPEVQMIRREANESSRFIGDDWHTDSTFLDAPPAAVVMRAIEVPEYGGDTGFLSMYSAWETLSPTMQATIEGLNVVHSATKVFGSLYQATNWRFSNTSVKVMDVDAGDRETVHPLVVTHPVTGRRALYCNQVYCQKIQGMTDAESKSLLQFLYEHATKFDFTCRVRWKKDQVLVWDNLCTMHRAVPDYAGKFRYLTRTTVAGDKPSR

SEQ ID NO: 15 - DNA, 906 bp, Artificial Sequence
  Recombinant
atgcacgcggctctgaccccgcttaccaacaaataccgtttcatcgacgttcagccgctgaccggtgttttaggtgctgaaatcaccggtgttgacctgcgtgaaccgctggacgactctacctggaacgaaatcctggacgcgttccacacctaccaggttatctacttcccgggtcaggcgatcaccaacgaacagcacatcgcgttctctcgtcgcttcggtccggttgacccggttccgattctcaaatctatcgaaggttacccggaagttcagatgatccgtcgcgaagcgaacgaatctagccgttttattggtgacgattggcacaccgactccaccttcctggacgcgccgccagctgcagttgtgatgcgtgctattgaagttccggaatacggtggcgacaccggtttcctgtccatgtactctgcttgggaaaccctgtccccgaccatgcaggctaccattgaaggtctgaacgttgtgcactccgcaaccaaagtgttcggcagcctgtaccaggcaaccaactggcgcttcagcaacactagtgtgaaagtgatggatgtggatgcaggcgatcgtgagactgtgcacccgctggtggtaactcacccggttaccggccgtcgtgcgctgtactgcaaccaggtatattgccagaaaattcagggcatgactgatgcagagtcaaaatctctgctccaatttctgtatgagcacgccactaaatttgattttacttgccgtgtccgttggaaaaaggatcaagtactggtatgggataatctgtgtacgatgcaccgcgccgtacctgattatgccggcaaatttcgctatttgacgcgcacgacagtcgcgggggacaaaccttctcgccatcaccatcatcatcattag

SEQ ID NO: 16 - DNA, 888 bp, Artificial Sequence
  Recombinant
atgcacgcggcgctgactcctctcaccaacaagtatcgctttatcgacgtgcagccgctgacaggcgtcctcggtgcagagattacaggcgtggatctgcgggagcctctcgatgacagcacttggaatgagatcctggacgcctttcacacctaccaagtgatctactttccgggtcaagctatcactaacgagcagcacatcgcgttctcccgccggttcggccctgtggacccggtgccgatcttaaagagtatcgagggctatccagaggtgcagatgatacggcgcgaggcgaacgagagcagccggttcatcggagatgactggcacaccgattccaccttcctggacgctccgcctgccgccgtggtgatgagagctatcgaagtgccggagtatggaggtgacacaggcttcctctccatgtacagtgcctgggagacactctcgcctacgatgcaagctaccatcgaaggcttaaacgtggtccactcggcgacgaaggtcttcgggtcattgtaccaggcgactaattggcgcttctcgaacaccagcgtgaaagtgatggacgtggacgccggagatagagagactgtgcacccactcgtcgtgacgcatcctgttacgggaaggcgcgcactctactgcaaccaggtgtactgccagaagatccagggaatgacggacgcggagtcgaagtccctgttgcaattcctttacgagcacgccaccaagttcgacttcacctgccgggtccggtggaagaaggaccaagtcctggtgtgggacaacctgtgtaccatgcaccgcgccgtcccggactacgctgggaaattcagatacctgacccgcaccaccgtggcgggagacaagccgtcgcgttga

SEQ ID NO: 17 - DNA, 888 bp, Artificial Sequence
  Recombinant
atgcacgcggctttgacacctttgaccaacaagtatcggttcatcgacgttcaaccactcacaggcgtgctcggcgcagagattaccggagtggacctgagggagcccttagacgactccacttggaacgagatcctcgacgcctttcacacctaccaagttatctactttcctggacaggcgatcaccaacgagcagcacattgccttctcaaggaggttcggaccggtagatccagttccaattctcaaatccattgagggttatcccgaggtgcagatgattagacgagaagccaacgagtcctcacggttcataggcgacgattggcacacagacagcaccttccttgacgctcctccggctgccgtggttatgcgcgcaatagaggtgccggagtacggcggcgataccggtttcctatcaatgtactctgcatgggagacgctctcaccaacgatgcaagccaccattgaaggtctaaacgtggttcactcagctactaaggtcttcggaagtctttaccaggcgacgaattggaggttcagtaacaccagtgtgaaggtgatggatgtggacgctggagacagggagacggtgcatccactcgtagttacacaccctgtaactggacgcagagccctttactgcaaccaggtttactgccagaagatccagggaatgactgatgcggagtctaagtccctgcttcaattcctctacgaacacgccaccaaattcgacttcacttgtcgtgttcggtggaagaaggaccaagtgctcgtgtgggataacctttgcaccatgcaccgagcagtaccagactacgccgggaaattccgctatctcacccgcactacagtggccggagacaagcctagccgctga

SEQ ID NO: 18 - protein, 295 aa, Artificial Sequence
  Recombinant
MHAALTPLTNKYRFIDVQPLTGVLGAEITGVDLREPLDDSTWNEILDAFHTYQVIYFPGQAITNEQHIAFSRRFGPVDPVPLLKSIEGYPEVQMIRREANESSRVIGDDWHSDSTFLDAPPAAVVMRAIEVPEYGGDTGFLSMYSAWETLSPTMQATIEGLNVVHSATKVFGSLYQATNWRFSNTSVKVMDVDAGDRETVHPLVVTHPVTGRRALYCNQVYCQKIQGMTDAESKSLLQFLYEHATKFDFTCRVRWKKDQVLVWDNLCTMHRAAPDYAGKFRYLTRTTVAGDKPSR

SEQ ID NO: 19 - DNA, 906 bp, Artificial Sequence
  Recombinant
atgcacgcggctctgaccccgcttaccaacaaataccgtttcatcgacgttcagccgctgaccggtgttttaggtgctgaaatcaccggtgttgacctgcgtgaaccgctggacgactctacctggaacgaaatcctggacgcgttccacacctaccaggttatctacttcccgggtcaggcgatcaccaacgaacagcacatcgcgttctctcgtcgcttcggtccggttgacccggttccgctgctcaaatctatcgaaggttacccggaagttcagatgatccgtcgcgaagcgaacgaatctagccgtgttattggtgacgattggcacagcgactccaccttcctggacgcgccgccagctgcagttgtgatgcgtgctattgaagttccggaatacggtggcgacaccggtttcctgtccatgtactctgcttgggaaaccctgtccccgaccatgcaggctaccattgaaggtctgaacgttgtgcactccgcaaccaaagtgttcggcagcctgtaccaggcaaccaactggcgcttcagcaacactagtgtgaaagtgatggatgtggatgcaggcgatcgtgagactgtgcacccgctggtggtaactcacccggttaccggccgtcgtgcgctgtactgcaaccaggtatattgccagaaaattcagggcatgactgatgcagagtcaaaatctctgctccaatttctgtatgagcacgccactaaatttgattttacttgccgtgtccgttggaaaaaggatcaagtactggtatgggataatctgtgtacgatgcaccgcgccgcgcctgattatgccggcaaatttcgctatttgacgcgcacgacagtcgcgggggacaaaccttctcgccatcaccatcatcatcattag

SEQ ID NO: 20 - DNA, 888 bp, Artificial Sequence
  Recombinant
atgcacgcggcgctgactcctctcaccaacaagtatcgctttatcgacgtgcagccgctgacaggcgtcctcggtgcagagattacaggcgtggatctgcgggagcctctcgatgacagcacttggaatgagatcctggacgcctttcacacctaccaagtgatctactttccgggtcaagctatcactaacgagcagcacatcgcgttctcccgccggttcggccctgtggacccggtgccgctgttaaagagtatcgagggctatccagaggtgcagatgatacggcgcgaggcgaacgagagcagccgggtgatcggagatgactggcactccgattccaccttcctggacgctccgcctgccgccgtggtgatgagagctatcgaagtgccggagtatggaggtgacacaggcttcctctccatgtacagtgcctgggagacactctcgcctacgatgcaagctaccatcgaaggcttaaacgtggtccactcggcgacgaaggtcttcgggtcattgtaccaggcgactaattggcgcttctcgaacaccagcgtgaaagtgatggacgtggacgccggagatagagagactgtgcacccactcgtcgtgacgcatcctgttacgggaaggcgcgcactctactgcaaccaggtgtactgccagaagatccagggaatgacggacgcggagtcgaagtccctgttgcaattcctttacgagcacgccaccaagttcgacttcacctgccgggtccggtggaagaaggaccaagtcctggtgtgggacaacctgtgtaccatgcaccgcgccgccccggactacgctgggaaattcagatacctgacccgcaccaccgtggcgggagacaagccgtcgcgttga

SEQ ID NO: 21 - DNA, 888 bp, Artificial Sequence
  Recombinant
atgcacgcagcccttactccactgacgaacaagtatcgcttcatcgacgtgcagccactcacgggtgtactcggagccgagatcacgggagtggatctgcgcgagccgctcgatgactctacatggaacgagatcctagacgctttccacacttatcaagttatctactttccaggacaagccatcactaacgagcaacacatcgcgttctcacgtcggttcgggcctgttgatcctgtgccgctcctcaagtcaatcgagggttatccagaagttcagatgatccggcgcgaggctaatgagtcatcccgtgttatcggtgatgactggcactcggacagtacattcctcgacgcaccaccggccgcagttgtgatgagggctatcgaagtgccggaatacggtggtgacactgggttcctgtcaatgtactctgcatgggagacccttagtcccactatgcaagcaaccatcgaagggctcaacgttgtgcattcagctactaaagtattcggttccctttatcaggcgacaaactggcggttcagcaataccagtgttaaagttatggatgtggatgctggagacagggaaacggtccaccctcttgtcgtcacgcacccagttacagggcgtcgagcgctttactgcaatcaggtgtactgtcagaagattcaaggaatgaccgatgcggagtccaaatcactgttacaattcttgtacgagcacgccactaagttcgatttcacgtgccgagtgcgctggaagaaggatcaagtgctcgtttgggacaacttgtgcaccatgcaccgggcagctcccgactacgcgggcaagttccgttatctcactcgcacaactgtcgctggagacaagccctcccgatga

SEQ ID NO: 22 - protein, 295 aa, Artificial Sequence
  Recombinant
MHAALSPLSQRFERIAVQPLTGVLGAEITGVDLREPLDDSTWNEILDAFHTYQVIYFPGQAITNEQHIAFSRRFGPVDPVPLLKSIEGYPEVQMIRREANESGRVIGDDWHTDSTFLDAPPAAVVMYAKEVPPYGGDTLFASMYTAWETLSPTMQATIEGLNVVHSATRVFGSLYQAQNRRFSNTSVKVMDVDAGDRETVHPLVVTHPETGRKGLYVNQVYCQRIEGMSEKESEPLLSFLFAHATKPEFTCRVRWQEGQVLVWDNLCTQHFAVPDYAGKFRYLTRTTVGGVRPAR

SEQ ID NO: 23 - DNA, 906 bp, Artificial Sequence
  Recombinant
atgcacgcggctctgagcccgcttagccagcgtttcgaacgtatcgcggttcagccgctgaccggtgttttaggtgctgaaatcaccggtgttgacctgcgtgaaccgctggacgactctacctggaacgaaatcctggacgcgttccacacctaccaggttatctacttcccgggtcaggcgatcaccaacgaacagcacatcgcgttctctcgtcgcttcggtccggttgacccggttccgctgctcaaatctatcgaaggttacccggaagttcagatgatccgtcgcgaagcgaacgaatctggtcgtgttattggtgacgactggcacaccgactctaccttcctggacgcgccgccagctgcagttgtgatgtacgctaaagaagtgccgccatacggtggcgacaccctgttcgcgtccatgtacaccgcttgggaaaccctgtccccgaccatgcaggctaccattgaaggtctgaacgttgtgcactccgcaactcgtgttttcggctccctgtaccaggcacagaaccgtcgcttcagcaacactagcgttaaagtgatggatgtggatgcaggcgatcgtgaaactgtgcacccgctggtggtaactcacccggaaactggccgtaaaggcctgtacgtgaaccaggtatattgccagcgtattgaaggcatgagtgagaaagagtcggagccgctgctctcatttctgtttgcacacgccactaaaccagagtttacttgccgtgtccgttggcaagagggccaggtactggtatgggataatctgtgtacgcaacacttcgccgtacctgattatgccggcaagtttcgctatttgacgcgcacgacagtcggcggggtccgccctgcccgccatcaccatcaccatcattag

SEQ ID NO: 24 - DNA, 888 bp, Artificial Sequence
  Recombinant
atgcacgcggccctgtctcctctgtcccagcggttcgagcgcatcgcggtccagccgctaacgggtgtcctgggcgcggaaatcaccggagttgatctgagagagcctttagacgacagcacctggaacgagatcctcgatgcctttcacacataccaagttatctactttcccggccaagccatcacgaacgagcagcacatcgcgtttagccggaggtttggcccggttgatccggttcctctgcttaagtcaattgagggttacccagaggtgcagatgatccgccgcgaggccaacgaatctgggcgtgtcataggcgacgattggcatacggacagcacctttctcgacgctcctccggccgcagtcgtgatgtacgcgaaggaggtgccgccttacggcggcgataccctgttcgcgtcgatgtacacggcctgggagacgctcagcccgaccatgcaagccacaatagagggtctaaatgtggtccactccgcgacgcgggtgttcgggagcctctaccaggcgcagaacagacggttctcgaacacatcagtcaaggtgatggacgtggatgccggagatcgtgaaactgttcacccacttgtggtcacccatccagagacgggaaggaaaggactttacgtgaaccaggtgtactgccagcggatcgagggcatgtccgagaaggagagtgagccattgctgagctttctattcgcgcacgcaactaagcccgagttcacgtgccgcgtccgatggcaagagggccaagttctcgtctgggataacttgtgcacacagcacttcgcggttcccgattacgccggaaagttccgctatctcacacgcaccactgtgggaggcgttcgtcccgcgcggtga

SEQ ID NO: 25 - protein, 295 aa, Artificial Sequence
  Recombinant
MHAALTPLTNKYRFIDVQPLTGVLGAEITGVDLREPLDDSTWNEILDAFHTYQVIYFPGQAITNEQHIAFSRRFGPVDPVPLLKSIEGYPEVQMIRREANESGRVIGDDWHTDSTFLDAPPAAVVMYAREVPPYGGDTGFLSMYTAWETLSPTMQATIEGLNVVHSATRVFGSLYQAQNRRYSNTSVKVMDVDAGDRETVHPLVVSHPVTGRRALYCNQVYCQRIEGMTDAESKSLLQFLYEHATKFDFTCRVRWKKDQVLVWDNLCTMHRAVPDYAGKFRYLTRTTVAGDKPSR

SEQ ID NO: 26 - DNA, 906 bp, Artificial Sequence
  Recombinant
atgcacgcggctctgaccccgcttaccaacaaataccgtttcatcgacgttcagccgctgaccggtgttttaggtgctgaaatcaccggtgttgacctgcgtgaaccgctggacgactctacctggaacgaaatcctggacgcgttccacacctaccaggttatctacttcccgggtcaggcgatcaccaacgaacagcacatcgcgttctctcgtcgcttcggtccggttgacccggttccgctgctcaaatctatcgaaggttacccggaagttcagatgatccgtcgcgaagcgaacgaatctggtcgtgttattggtgacgattggcacaccgactccaccttcctggacgcgccgccagctgcagttgtgatgtacgctcgtgaagttccgccgtacggtggcgacaccggtttcctgtccatgtacaccgcttgggaaaccctgtccccgaccatgcaggctaccattgaaggtctgaacgttgtgcactccgcaacccgtgtgttcggcagcctgtaccaggcacagaaccgtcgctacagcaacactagtgtgaaagtgatggatgtggatgcaggcgatcgtgagactgtgcacccgctggtggtatctcacccggttaccggccgtcgtgcgctgtactgcaaccaggtatattgccagcgtattgagggcatgactgatgcagagtcaaaatctctgctccaatttctgtatgagcacgccactaaatttgattttacttgccgtgtccgttggaaaaaggatcaagtactggtatgggataatctgtgtacgatgcaccgcgccgtacctgattatgccggcaaatttcgctatttgacgcgcacgacagtcgcgggggacaaaccttctcgccatcaccatcatcatcattag

SEQ ID NO: 27 - DNA, 888 bp, Artificial Sequence
  Recombinant
atgcacgctgctctgactccactcacaaacaagtaccggttcatcgacgtgcaaccgctgaccggcgtcttgggtgcggaaatcaccggcgtggacttgcgggagccgctggatgacagcacatggaacgagatcctcgatgcgttccacacctaccaagtgatctatttcccaggccaggccattacgaacgagcagcacatcgcgttcagtcgaaggttcgggcctgtggacccggttccgctgcttaagagtatcgagggctacccggaagtacagatgattcgccgcgaagcgaatgagtccgggcgagtgatcggcgatgactggcacaccgacagcacgttcctcgacgcgccgcctgccgctgtcgtgatgtacgcacgggaggtgccaccctacggcggagatacgggattcctttcaatgtacacggcatgggagacactctctccgaccatgcaagcaacgatagagggcttgaacgtggtgcactccgccacgagggtcttcggcagcctctaccaagcccagaaccgccggtactccaacactagcgtgaaagtgatggacgtggatgcgggcgaccgggagaccgtgcatcctctagttgtgagccacccggtgactggccgacgggcgctgtactgcaaccaggtctattgccagcgcatcgagggcatgaccgacgcggagtcgaaatctctgctccaattcctgtacgagcacgccacgaagttcgacttcacctgccgggttcgctggaagaaggatcaagtgctagtgtgggacaacctctgcactatgcacagggctgtgccggactatgctggcaaattccgttaccttacccggaccactgtggcgggcgacaagccaagcagatga

SEQ ID NO: 28 - protein, 295 aa, Artificial Sequence
  Recombinant
MHAALTPLTNKYRFIDVQPLTGVLGAEITGVDLREPLDDSTWNEILDAFHTYQVIYFPGQAITNEQHIAFSRRFGPVDPVPLLKSIEGYPEVQMIRREANESGRVIGDDWHTDSTFLDAPPAAVVMRAIEVPEYGGDTGFLSMYSAWETLSPTMQATIEGLNVVHSATKVFGSLYQATNWRFSNTSVKVMDVDAGDRETVHPLVVTHPVTGRRALYCNQVYCQKIQGMTDAESKSLLQFLYEHATKFDFTCRVRWKKDQVLVWDNLCTMHRAVPDYAGKFRYLTRTTVAGDKPSR

SEQ ID NO: 29 - DNA, 906 bp, Artificial Sequence
  Recombinant
atgcacgcggctctgaccccgcttaccaacaaataccgtttcatcgacgttcagccgctgaccggtgttttaggtgctgaaatcaccggtgttgacctgcgtgaaccgctggacgactctacctggaacgaaatcctggacgcgttccacacctaccaggttatctacttcccgggtcaggcgatcaccaacgaacagcacatcgcgttctctcgtcgcttcggtccggttgacccggttccgctgctcaaatctatcgaaggttacccggaagttcagatgatccgtcgcgaagcgaacgaatctggtcgtgttattggtgacgattggcacaccgactccaccttcctggacgcgccgccagctgcagttgtgatgcgtgctattgaagttccggaatacggtggcgacaccggtttcctgtccatgtactctgcttgggaaaccctgtccccgaccatgcaggctaccattgaaggtctgaacgttgtgcactccgcaaccaaagtgttcggcagcctgtaccaggcaaccaactggcgcttcagcaacactagtgtgaaagtgatggatgtggatgcaggcgatcgtgagactgtgcacccgctggtggtaactcacccggttaccggccgtcgtgcgctgtactgcaaccaggtatattgccagaaaattcagggcatgactgatgcagagtcaaaatctctgctccaatttctgtatgagcacgccactaaatttgattttacttgccgtgtccgttggaaaaaggatcaagtactggtatgggataatctgtgtacgatgcaccgcgccgtacctgattatgccggcaaatttcgctatttgacgcgcacgacagtcgcgggggacaaaccttctcgccatcaccatcatcatcattag

SEQ ID NO: 30 - DNA, 888 bp, Artificial Sequence
  Recombinant
atgcacgcggcgctgactcctctcaccaacaagtatcgctttatcgacgtgcagccgctgacaggcgtcctcggtgcagagattacaggcgtggatctgcgggagcctctcgatgacagcacttggaatgagatcctggacgcctttcacacctaccaagtgatctactttccgggtcaagctatcactaacgagcagcacatcgcgttctcccgccggttcggccctgtggacccggtgccgctgttaaagagtatcgagggctatccagaggtgcagatgatacggcgcgaggcgaacgagagcggccgggtgatcggagatgactggcacaccgattccaccttcctggacgctccgcctgccgccgtggtgatgagagctatcgaagtgccggagtatggaggtgacacaggcttcctctccatgtacagtgcctgggagacactctcgcctacgatgcaagctaccatcgaaggcttaaacgtggtccactcggcgacgaaggtcttcgggtcattgtaccaggcgactaattggcgcttctcgaacaccagcgtgaaagtgatggacgtggacgccggagatagagagactgtgcacccactcgtcgtgacgcatcctgttacgggaaggcgcgcactctactgcaaccaggtgtactgccagaagatccagggaatgacggacgcggagtcgaagtccctgttgcaattcctttacgagcacgccaccaagttcgacttcacctgccgggtccggtggaagaaggaccaagtcctggtgtgggacaacctgtgtaccatgcaccgcgccgtcccggactacgctgggaaattcagatacctgacccgcaccaccgtggcgggagacaagccgtcgcgttga

SEQ ID NO: 31 - protein, 295 aa, Artificial Sequence
  Recombinant
MHAALSPLSQKYRFIDVQPLTGVLGAEITGVTLREPLDDNTWNEILDAFHTYQVIYFPGQAITNEQHIAFSRRFGPVDPVPLLKSIEGYPEVQMIRREANESGRVIGDDWHTDSTFLDAPPAAVVMYAREVPPYGGDTGFLSMYSAWDTLSDTMKATIEGLNVVHSATRVFGSLYQAQNRRFSNTSVKVMDVDAGDRETVHPLVVSHPVTGRRALYCNQVYCQRIEGMTDAESKPLLQFLYEHATRFDFTCRVRWKKDQVLVWDNLCTMHRAVPDYAGKFRYLTRTTVAGDKPSR

SEQ ID NO: 32 - DNA, 906 bp, Artificial Sequence
  Recombinant
atgcacgcggctctgagcccgcttagccagaaataccgtttcatcgacgttcagccgctgaccggtgttttaggtgctgaaatcaccggtgttaccctgcgtgaaccgctggacgacaacacctggaacgaaatcctggacgcgttccacacctaccaggttatctacttcccgggtcaggcgatcaccaacgaacagcacatcgcgttctctcgtcgcttcggtccggttgacccggttccgctgctcaaatctatcgaaggttacccggaagttcagatgatccgtcgcgaagcgaacgaatctggtcgtgttattggtgacgattggcacaccgactccaccttcctggacgcgccgccagctgcagttgtgatgtacgctcgtgaagttccgccgtacggtggcgacaccggtttcctgtccatgtactctgcttgggacaccctgtccgacaccatgaaagctaccattgaaggtctgaacgttgtgcactccgcaacccgtgtgttcggcagcctgtaccaggcacagaaccgtcgcttcagcaacactagtgtgaaagtgatggatgtggatgcaggcgatcgtgagactgtgcacccgctggtggtatctcacccggttaccggccgtcgtgcgctgtactgcaaccaggtatattgccagcgtattgagggcatgactgatgcagagtcaaaaccactgctccaatttctgtatgagcacgccactcgttttgattttacttgccgtgtccgttggaaaaaggatcaagtactggtatgggataatctgtgtacgatgcaccgcgccgtacctgattatgccggcaaatttcgctatttgacgcgcacgacagtcgcgggggacaaaccttctcgccatcaccatcatcatcattag

SEQ ID NO: 33 - DNA, 888 bp, Artificial Sequence
  Recombinant
atgcacgccgccctctctcctcttagccagaagtaccgattcatcgacgtccagccgctcactggcgtactgggcgctgagataacgggtgtgaccctgagggagccgctggacgacaacacttggaacgagatccttgacgccttccatacttatcaagttatctactttcctggacaagcgattacgaatgagcagcacatcgcgttctcccggaggttcgggccagtcgatccggtgccgctactcaagtccatcgaaggatacccagaagtccagatgatccgtcgtgaggcaaacgagtccggccgggtcatcggcgacgattggcacaccgactctaccttccttgacgcgcctccggccgcagtggtcatgtacgcccgcgaggtgcctccctacggcggcgatacgggcttcctcagtatgtactctgcatgggacaccctaagcgacaccatgaaggccaccatcgaaggtctgaacgtcgtgcactcggcaacacgagtcttcggatcactctaccaagcacagaatcgccgcttctcgaacacctcggttaaggtgatggacgtggatgcgggtgacagggaaaccgttcatcctctggtggtctcgcatccggttacgggacgccgcgctctctactgcaaccaggtgtactgtcaaaggatcgaaggaatgacagatgctgagagcaagccgttgctccaattcctctatgaacacgcaacaaggttcgacttcacctgccgggttcgatggaagaaggatcaagtgctagtctgggacaacctctgcaccatgcaccgggccgtgccggactatgctgggaaattccgttacctgacccgcacgaccgtcgcgggagacaagccgtcgagatga

SEQ ID NO: 34 - protein, 295 aa, Artificial Sequence
  Recombinant
MHAALTPLTNKYRFIDVQPLTGVLGAEITGVDLREPLDDSTWNEILDAFHTYQVIYFPGQAITNEQHIAFSRRFGPVDPVPLLKSIEGYPEVQMIRREANESGRVIGDDWHADSTFLDAPPAAVVMRAIEVPEYGGDTGFLSMYSAWETLSPTMQATIEGLNVVHSATKVFGSLYQATNWRFSNTSVKVMDVDAGDRETVHPLVVTHPVTGRRALYCNQVYCQKIQGMTDAESKSLLQFLYEHATKFDFTCRVRWKKDQVLVWDNLCTMHRSVPDYAGKFRYLTRTTVAGDKPSR

SEQ ID NO: 35 - DNA, 906 bp, Artificial Sequence
  Recombinant
atgcacgcggctctgaccccgcttaccaacaaataccgtttcatcgacgttcagccgctgaccggtgttttaggtgctgaaatcaccggtgttgacctgcgtgaaccgctggacgactctacctggaacgaaatcctggacgcgttccacacctaccaggttatctacttcccgggtcaggcgatcaccaacgaacagcacatcgcgttctctcgtcgcttcggtccggttgacccggttccgctgctcaaatctatcgaaggttacccggaagttcagatgatccgtcgcgaagcgaacgaatctggtcgtgttattggtgacgattggcacgcggactccaccttcctggacgcgccgccagctgcagttgtgatgcgtgctattgaagttccggaatacggtggcgacaccggtttcctgtccatgtactctgcttgggaaaccctgtccccgaccatgcaggctaccattgaaggtctgaacgttgtgcactccgcaaccaaagtgttcggcagcctgtaccaggcaaccaactggcgcttcagcaacactagtgtgaaagtgatggatgtggatgcaggcgatcgtgagactgtgcacccgctggtggtaactcacccggttaccggccgtcgtgcgctgtactgcaaccaggtatattgccagaaaattcagggcatgactgatgcagagtcaaaatctctgctccaatttctgtatgagcacgccactaaatttgattttacttgccgtgtccgttggaaaaaggatcaagtactggtatgggataatctgtgtacgatgcaccgcagcgtacctgattatgccggcaaatttcgctatttgacgcgcacgacagtcgcgggggacaaaccttctcgccatcaccatcatcatcattag

SEQ ID NO: 36 - DNA, 888 bp, Artificial Sequence
  Recombinant
atgcacgcggcgctgactcctctcaccaacaagtatcgctttatcgacgtgcagccgctgacaggcgtcctcggtgcagagattacaggcgtggatctgcgggagcctctcgatgacagcacttggaatgagatcctggacgcctttcacacctaccaagtgatctactttccgggtcaagctatcactaacgagcagcacatcgcgttctcccgccggttcggccctgtggacccggtgccgctgttaaagagtatcgagggctatccagaggtgcagatgatacggcgcgaggcgaacgagagcggccgggtgatcggagatgactggcacgccgattccaccttcctggacgctccgcctgccgccgtggtgatgagagctatcgaagtgccggagtatggaggtgacacaggcttcctctccatgtacagtgcctgggagacactctcgcctacgatgcaagctaccatcgaaggcttaaacgtggtccactcggcgacgaaggtcttcgggtcattgtaccaggcgactaattggcgcttctcgaacaccagcgtgaaagtgatggacgtggacgccggagatagagagactgtgcacccactcgtcgtgacgcatcctgttacgggaaggcgcgcactctactgcaaccaggtgtactgccagaagatccagggaatgacggacgcggagtcgaagtccctgttgcaattcctttacgagcacgccaccaagttcgacttcacctgccgggtccggtggaagaaggaccaagtcctggtgtgggacaacctgtgtaccatgcaccgctccgtcccggactacgctgggaaattcagatacctgacccgcaccaccgtggcgggagacaagccgtcgcgttga

SEQ ID NO: 37 - protein, 295 aa, Artificial Sequence
  Recombinant
MHAALTPLTNKYRFIDVQPLTGVLGAEITGVDLREPLDDSTWNEILDAFHTYQVIYFPGQAITNEQHIAFSRRFGPVDPVPILKSIEGYPEVQMIRREANESGRVIGDDWHTDSTFLDAPPAAVVMRAIEVPEYGGDTGFLSMYSAWETLSPTMQATIEGLNVVHSATKVFGSLYQATNWRFSNTSVKVMDVDAGDRETVHPLVVTHPVTGRRALYCNQVYCQKIQGMTDAESKSLLQFLYEHATKFDFTCRVRWKKDQVLVWDNLCTMHRSVPDYGNAFRYLTRTTVAGDKPSR

SEQ ID NO: 38 - DNA, 906 bp, Artificial Sequence
  Recombinant
atgcacgcggctctgaccccgcttaccaacaaataccgtttcatcgacgttcagccgctgaccggtgttttaggtgctgaaatcaccggtgttgacctgcgtgaaccgctggacgactctacctggaacgaaatcctggacgcgttccacacctaccaggttatctacttcccgggtcaggcgatcaccaacgaacagcacatcgcgttctctcgtcgcttcggtccggttgacccggttccgattctcaaatctatcgaaggttacccggaagttcagatgatccgtcgcgaagcgaacgaatctggtcgtgttattggtgacgattggcacaccgactccaccttcctggacgcgccgccagctgcagttgtgatgcgtgctattgaagttccggaatacggtggcgacaccggtttcctgtccatgtactctgcttgggaaaccctgtccccgaccatgcaggctaccattgaaggtctgaacgttgtgcactccgcaaccaaagtgttcggcagcctgtaccaggcaaccaactggcgcttcagcaacactagtgtgaaagtgatggatgtggatgcaggcgatcgtgagactgtgcacccgctggtggtaactcacccggttaccggccgtcgtgcgctgtactgcaaccaggtatattgccagaaaattcagggcatgactgatgcagagtcaaaatctctgctccaatttctgtatgagcacgccactaaatttgattttacttgccgtgtccgttggaaaaaggatcaagtactggtatgggataatctgtgtacgatgcaccgcagcgtacctgattatggcaatgcgtttcgctatttgacgcgcacgacagtcgcgggggacaaaccttctcgccatcaccatcatcatcattag

SEQ ID NO: 39 - DNA, 888 bp, Artificial Sequence
  Recombinant
atgcacgcggcgctgactcctctcaccaacaagtatcgctttatcgacgtgcagccgctgacaggcgtcctcggtgcagagattacaggcgtggatctgcgggagcctctcgatgacagcacttggaatgagatcctggacgcctttcacacctaccaagtgatctactttccgggtcaagctatcactaacgagcagcacatcgcgttctcccgccggttcggccctgtggacccggtgccgatcttaaagagtatcgagggctatccagaggtgcagatgatacggcgcgaggcgaacgagagcggccgggtgatcggagatgactggcacaccgattccaccttcctggacgctccgcctgccgccgtggtgatgagagctatcgaagtgccggagtatggaggtgacacaggcttcctctccatgtacagtgcctgggagacactctcgcctacgatgcaagctaccatcgaaggcttaaacgtggtccactcggcgacgaaggtcttcgggtcattgtaccaggcgactaattggcgcttctcgaacaccagcgtgaaagtgatggacgtggacgccggagatagagagactgtgcacccactcgtcgtgacgcatcctgttacgggaaggcgcgcactctactgcaaccaggtgtactgccagaagatccagggaatgacggacgcggagtcgaagtccctgttgcaattcctttacgagcacgccaccaagttcgacttcacctgccgggtccggtggaagaaggaccaagtcctggtgtgggacaacctgtgtaccatgcaccgctccgtcccggactacggcaacgccttcagatacctgacccgcaccaccgtggcgggagacaagccgtcgcgttga

SEQ ID NO: 40 - protein, 295 aa, Artificial Sequence
  Recombinant
MHAALTPLTNKYRFIDVQPLTGVLGAEITGVDLREPLDDSTWNEILDAFHTYQVIYFPAQQITNEQHISFSRRFGPVDPVPLLKSIEGYPEVQMIRREANESGRILGDDWHTDSTFLDAPPAAVVMRAIEVPEYGGDTGFLSMYSAWDTLSDTMKATIEGLNVVHSATRVFGSLYQAQNWRFSNTSVKVMDVDAGDRETVHPLVVSHPVTGRRALYCNQVYCQRIEGMTDAESKCLLQFLYEHATKFDFTCRVRWKKDQVLVWDNLCTMHRAVPDYAGKFRYLTRTTVAGDRPAR

SEQ ID NO: 41 - DNA, 906 bp, Artificial Sequence
  Recombinant
atgcacgcggctctgaccccgcttaccaacaaataccgtttcatcgacgttcagccgctgaccggtgttttaggtgctgaaatcaccggtgttgacctgcgtgaaccgctggacgactctacctggaacgaaatcctggacgcgttccacacctaccaggttatctacttcccggcgcagcagatcaccaacgaacagcacatctctttctctcgtcgcttcggtccggttgacccggttccgctgctcaaatctatcgaaggttacccggaagttcagatgatccgtcgcgaagcgaacgaatctggtcgtatcctgggtgacgattggcacaccgactccaccttcctggacgcgccgccagctgcagttgtgatgcgtgctattgaagttccggaatacggtggcgacaccggtttcctgtccatgtactctgcttgggacaccctgtccgacaccatgaaagctaccattgaaggtctgaacgttgtgcactccgcaacccgtgtgttcggcagcctgtaccaggcacagaactggcgcttcagcaacactagtgtgaaagtgatggatgtggatgcaggcgatcgtgagactgtgcacccgctggtggtatctcacccggttaccggccgtcgtgcgctgtactgcaaccaggtatattgccagcgtattgagggcatgactgatgcagagtcaaaatgcctgctccaatttctgtatgagcacgccactaaatttgattttacttgccgtgtccgttggaaaaaggatcaagtactggtatgggataatctgtgtacgatgcaccgcgccgtacctgattatgccggcaaatttcgctatttgacgcgcacgacagtcgcgggggaccgccctgcccgccatcaccatcatcatcattag

SEQ ID NO: 42 - DNA, 888 bp, Artificial Sequence
  Recombinant
atgcacgccgccttaacgccactcacgaacaagtatcgcttcatcgacgtccagccgctcactggcgtgctaggtgctgagatcaccggcgttgatctccgcgagcctcttgacgactcgacctggaacgagatcctggatgccttccacacttaccaagtgatctacttcccggcccaacagatcacaaacgagcagcacatctcctttagtaggcgattcggtccagtcgatccggtgccgctcctcaagtcgattgagggctacccggaggtccagatgattcgtagggaagccaacgagtcaggccgtattctgggcgacgactggcatacggactccactttcctagacgcacctccggctgccgtcgtcatgagggctattgaagtgccggagtacggcggcgataccggattcctctctatgtactccgcctgggacacgctctcagacaccatgaaggccacgatagagggcctgaacgttgtgcactccgcaacgagagtattcggatctctgtaccaggcacagaactggcggttcagtaacacgagcgtgaaagtcatggacgtggacgctggcgacagggaaactgttcacccgttggtcgtttcccaccctgtcactggtcgccgggcactttactgcaaccaggtgtactgtcagcgcattgagggcatgacggatgctgagtcgaagtgccttctccaattcttgtacgagcacgcgacaaagttcgatttcacgtgccgggtccgatggaagaaggaccaagtgctagtgtgggacaacctttgcacgatgcaccgcgctgtcccggattacgccggaaagttccgttacctcaccagaacaacagttgccggtgacagacccgcgagatga

SEQ ID NO: 43 - protein, 295 aa, Artificial Sequence
  Recombinant
MHAALTPLTNKYRFIDVQPLCGVLGAEITGVDLREPLDDSTWNEILDAFHTYQVIYFPGQAITNEQHIAFSRRFGPVDPVPLLKSIEGYPEVQMIRREANESGRILGDDWHTDSTFLDAPPAAVVMRAIEVPEYGGDTGFLSMYSAWDTLSDTMKATIEGLNVVHSATRVFGSLYQAQNWRFSNTSVKVMDVDAGDRETVHPLVVSHPVTGRRALYCNQVYCQRIEGMTDAESKCLLQFLYEHATKFDFTCRVRWKKDQVLVWDNLCTMHLAVPDYDGKFRYLTRTTVAGDKPSR

SEQ ID NO: 44 - DNA, 906 bp, Artificial Sequence
  Recombinant
atgcacgcggctctgaccccgcttaccaacaaataccgtttcatcgacgttcagccgctgtgcggtgttttaggtgctgaaatcaccggtgttgacctgcgtgaaccgctggacgactctacctggaacgaaatcctggacgcgttccacacctaccaggttatctacttcccgggtcaggcgatcaccaacgaacagcacatcgcgttctctcgtcgcttcggtccggttgacccggttccgctgctcaaatctatcgaaggttacccggaagttcagatgatccgtcgcgaagcgaacgaatctggtcgtatcctgggtgacgattggcacaccgactccaccttcctggacgcgccgccagctgcagttgtgatgcgtgctattgaagttccggaatacggtggcgacaccggtttcctgtccatgtactctgcttgggacaccctgtccgacaccatgaaagctaccattgaaggtctgaacgttgtgcactccgcaacccgtgtgttcggcagcctgtaccaggcacagaactggcgcttcagcaacactagtgtgaaagtgatggatgtggatgcaggcgatcgtgagactgtgcacccgctggtggtatctcacccggttaccggccgtcgtgcgctgtactgcaaccaggtatattgccagcgtattgagggcatgactgatgcagagtcaaaatgcctgctccaatttctgtatgagcacgccactaaatttgattttacttgccgtgtccgttggaaaaaggatcaagtactggtatgggataatctgtgtacgatgcacctggccgtacctgattatgacggcaaatttcgctatttgacgcgcacgacagtcgcgggggacaaaccttctcgccatcaccatcatcatcattag

SEQ ID NO: 45 - DNA, 888 bp, Artificial Sequence
  Recombinant
atgcacgcggctctcacaccgctcacaaacaagtaccgcttcattgacgtgcagccgctgtgtggcgtcctgggcgcagaaatcacgggcgtggatctccgcgagcctctggacgacagcacctggaacgaaatcctggatgctttccacacttaccaagtgatctactttcccggacaagccatcactaacgagcagcacatcgctttctcacggcgcttcggcccggtagatccggtgccgctactcaagtcaattgaaggctatccggaggtgcaaatgattcgccgcgaagctaacgagagcgggcgcatactgggcgacgactggcatactgactccaccttcctcgatgctccaccagccgcagtggtgatgcgtgccatcgaagttcccgagtatggtggcgacacgggtttcctgtctatgtactccgcttgggatacactgtctgacacgatgaaggctaccatcgagggcctgaatgtcgtccacagtgctacgcgcgtgttcggctcactgtaccaggcgcagaactggaggttcagcaacaccagtgtcaaggtgatggacgttgatgctggagacagggaaactgtgcatcctcttgtggtctcccatccagttaccgggaggagagcactctactgcaaccaggtttactgccagcgcatcgagggcatgaccgatgcggagtcgaagtgtctgttacagttcttgtacgagcacgcgacgaagttcgacttcacgtgccgggtgcggtggaagaaggaccaagttctcgtctgggacaatctctgcacgatgcacctcgccgttcccgactacgacggcaaattcagatacttgacccgaacaacagtagcgggagataagccttcccgttga

SEQ ID NO: 46 - protein, 295 aa, Artificial Sequence
  Recombinant
MHAALTPLTNKYRFIDVQPLTGVLGAEITGVDLREPLDDSTWNEILDAFHTYQVIYFPGQAITNEQHIAFSRRFGPVDPVPILKSIEGYPEVQMIRREANESSRYIGDDWHADSTFLDAPPAAVVMRAIEVPEYGGDTGFLSMYSAWETLSPTMQATIEGLNVVHSATKVFGSLYQATNWRFSNTSVKVMDVDAGDRETVHPLVVTHPVTGRRALYCNQVYCQKIQGMTDAESKSLLQFLYEHATKFDFTCRVRWKKDQVLVWDNLCTMHRAVPDYAGKFRYLTRTTVAGDKPSR

SEQ ID NO: 47 - protein, 295 aa, Artificial Sequence
  Recombinant
MHAALTPLTNKYRFIDVQPLTGVLGAEITGVDLREPLDDSTWNEILDAFHTYQVIYFPGQAITNEQHIAFSRRFGPVDPVPILKSIEGYPEVQMIRREANESSRYIGDDWHADSTFLDAPPAAVVMRAIEVPEYGGDTGFLSMYSAWETLSPTMQATIEGLNVVHSATKVFGSLYQATNWRFSGTSVKVMDVDAGDRETVHPLVVTHPVTGRRALYCNQVYCQKIQGMTDAESKSLLQFLYEHATQFDFTCRVRWKKDQVLVWDNLCTMHRAVPDYAGKFRYLTRTTVAGDKPSR

SEQ ID NO: 48 - protein, 295 aa, Artificial Sequence
  Recombinant
MHAALTPLTNKYRHIDVQPLTGVLGAEITGVDLREPLDDSTWNEILDAFHTYQVIYFPGQAITNEQHIAFSRRFGPVDPVPILKSIEGYPEVQMIRREANESSRYIGDDWHADSTFLDAPPAAVVMRAIEVPEYGGDTGFLSMYSAWETLSPTMQATIEGLNVVHSATKVFGSLYQATNWRFSGTSVKVMDVDAGDRETVHPLVVTHPVTGRRALYCNQVYCQKIQGMTDAESKSLLQFLYEHATQFDFTCRVRWKKDQVLVWDNLCTMHRAVPDYAGKFRYLTRTTVAGDKPSR

SEQ ID NO: 49 - protein, 295 aa, Artificial Sequence
  Recombinant
MHAALTPLTNKYRHIDVQPLTGVLGAEITGVDLREPLDDSTWNEILDAFHTYQVIYFPGQAITNEQHIAFSRRFGPVDPVPILKSIEGYPEVQMIRREANESSRYIGDDWHADSTFLDAPPAAVVMRAIEVPEYGGDTGFLSMYSAWETLSPAMQATIEGLNVVHSATKVFGSLYQATNWRFSNTSVKVMDVDAGDRETVHPLVVTHPVTGRRALYCNQIYCQKIQGMTDAESKSLLQFLYEHATQFDFTCRVRWKKDQVLVWDNLCTMHRAVPDYAGKFRYLTRTTVAGDKPSR

SEQ ID NO: 50 - protein, 295 aa, Artificial Sequence
  Recombinant
MHAALTPLTNKYRFIDVQPLTGVLGAEITGVDLREPLDDSTWNEILDAFHTYQVIYFPGQAITNEQHIAFSRRFGPVDPVPILKSIEGYPEVQMIRREANESSRYIGDDWHADSTFLDAPPAAVVMRAIEVPEYGGDTGFLSMYSAWETLSPTMQATIEGLNVVHSATKVFGSLYQATNWRFSNTSVKVMDVDAGDRETVHPLVVTHPVTGRRALYCNQIYCQKIQGMTDAESKSLLQFLYEHATQFDFTCRVRWKKDQVLVWDNLCTMHRAVPDYAGKFRYLTRTTVAGDKPSR

SEQ ID NO: 51 - protein, 295 aa, Artificial Sequence
  Recombinant
MHAALTPLTNKYRFIDVQPLTGVLGAEITGVDLREPLDDSTWNEILDAFHTYQVIYFPGQAITNEQHIAFSRRFGPVDPVPILKSIEGYPEVQMIRREANESSRYIGDDWHADSTFLDAPPAAVVMRAIEVPEYGGDTGFLSMYSAWETLSPTMQATIEGLNVVHSATKVFGSLYQATNWRFSNTSVKVMDVDAGDRETVHPLVVTHPVTGRRALYCNQVYCQKIQGMTDAESKSLLQFLYEHATQFDFTCRVRWKKDQVLVWDNLCTMHRAVPDYAGKFRYLTRTTVAGDKPSR

SEQ ID NO: 52 - protein, 295 aa, Artificial Sequence
  Recombinant
MHAALTPLTNKYRHIDVQPLTGVLGAEITGVDLREPLDDSTWNEILDAFHTYQVIYFPGQAITNEQHIAFSRRFGPVDPVPILKSIEGYPEVQMIRREANESSRYIGDDWHADSTFLDAPPAAVVMRAIEVPEYGGDTGFLSMYSAWETLSPTMQATIEGLNVVHSATKVFGSLYQATNWRFSNTSVKVMDVDAGDRETVHPLVVTHPVTGRRALYCNQVYCQKIQGMTDAESKSLLQFLYEHATQFDFTCRVRWKKDQVLVWDNLCTMHRAVPDYAGKFRYLTRTTVAGDKPSR

SEQ ID NO: 53 - DNA, 888 bp, Artificial Sequence
  Recombinant
atgcacgcggctttgacacctttgaccaacaagtatcggttcatcgacgttcaaccactcacaggcgtgctcggcgcagagattaccggagtggacctgagggagcccttagacgactccacttggaacgagatcctcgacgcctttcacacctaccaagttatctactttcctggacaggcgatcaccaacgagcagcacattgccttctcaaggaggttcggaccggtagatccagttccaattctcaaatccattgagggttatcccgaggtgcagatgattagacgagaagccaacgagtcctcacggtacataggcgacgattggcacgcagacagcaccttccttgacgctcctccggctgccgtggttatgcgcgcaatagaggtgccggagtacggcggcgataccggtttcctatcaatgtactctgcatgggagacgctctcaccaacgatgcaagccaccattgaaggtctaaacgtggttcactcagctactaaggtcttcggaagtctttaccaggcgacgaattggaggttcagtaacaccagtgtgaaggtgatggatgtggacgctggagacagggagacggtgcatccactcgtagttacacaccctgtaactggacgcagagccctttactgcaaccaggtttactgccagaagatccagggaatgactgatgcggagtctaagtccctgcttcaattcctctacgaacacgccaccaaattcgacttcacttgtcgtgttcggtggaagaaggaccaagtgctcgtgtgggataacctttgcaccatgcaccgagcagtaccagactacgccgggaaattccgctatctcacccgcactacagtggccggagacaagcctagccgctga

SEQ ID NO: 54 - DNA, 888 bp, Artificial Sequence
  Recombinant
atgcacgcggctttgacacctttgaccaacaagtatcggttcatcgacgttcaaccactcacaggcgtgctcggcgcagagattaccggagtggacctgagggagcccttagacgactccacttggaacgagatcctcgacgcctttcacacctaccaagttatctactttcctggacaggcgatcaccaacgagcagcacattgccttctcaaggaggttcggaccggtagatccagttccaattctcaaatccattgagggttatcccgaggtgcagatgattagacgagaagccaacgagtcctcacggtacataggcgacgattggcacgcagacagcaccttccttgacgctcctccggctgccgtggttatgcgcgcaatagaggtgccggagtacggcggcgataccggtttcctatcaatgtactctgcatgggagacgctctcaccaacgatgcaagccaccattgaaggtctaaacgtggttcactcagctactaaggtcttcggaagtctttaccaggcgacgaattggaggttcagtggaaccagtgtgaaggtgatggatgtggacgctggagacagggagacggtgcatccactcgtagttacacaccctgtaactggacgcagagccctttactgcaaccaggtttactgccagaagatccagggaatgactgatgcggagtctaagtccctgcttcaattcctctacgaacacgccacccaattcgacttcacttgtcgtgttcggtggaagaaggaccaagtgctcgtgtgggataacctttgcaccatgcaccgagcagtaccagactacgccgggaaattccgctatctcacccgcactacagtggccggagacaagcctagccgctga

SEQ ID NO: 55 - DNA, 888 bp, Artificial Sequence
  Recombinant
atgcacgcggctttgacacctttgaccaacaagtatcggcatatcgacgttcaaccactcacaggcgtgctcggcgcagagattaccggagtggacctgagggagcccttagacgactccacttggaacgagatcctcgacgcctttcacacctaccaagttatctactttcctggacaggcgatcaccaacgagcagcacattgccttctcaaggaggttcggaccggtagatccagttccaattctcaaatccattgagggttatcccgaggtgcagatgattagacgagaagccaacgagtcctcacggtacataggcgacgattggcacgcagacagcaccttccttgacgctcctccggctgccgtggttatgcgcgcaatagaggtgccggagtacggcggcgataccggtttcctatcaatgtactctgcatgggagacgctctcaccaacgatgcaagccaccattgaaggtctaaacgtggttcactcagctactaaggtcttcggaagtctttaccaggcgacgaattggaggttcagtggaaccagtgtgaaggtgatggatgtggacgctggagacagggagacggtgcatccactcgtagttacacaccctgtaactggacgcagagccctttactgcaaccaggtttactgccagaagatccagggaatgactgatgcggagtctaagtccctgcttcaattcctctacgaacacgccacccaattcgacttcacttgtcgtgttcggtggaagaaggaccaagtgctcgtgtgggataacctttgcaccatgcaccgagcagtaccagactacgccgggaaattccgctatctcacccgcactacagtggccggagacaagcctagccgctga

SEQ ID NO: 56 - DNA, 888 bp, Artificial Sequence
  Recombinant
atgcacgcggctttgacacctttgaccaacaagtatcggcatatcgacgttcaaccactcacaggcgtgctcggcgcagagattaccggagtggacctgagggagcccttagacgactccacttggaacgagatcctcgacgcctttcacacctaccaagttatctactttcctggacaggcgatcaccaacgagcagcacattgccttctcaaggaggttcggaccggtagatccagttccaattctcaaatccattgagggttatcccgaggtgcagatgattagacgagaagccaacgagtcctcacggtacataggcgacgattggcacgcagacagcaccttccttgacgctcctccggctgccgtggttatgcgcgcaatagaggtgccggagtacggcggcgataccggtttcctatcaatgtactctgcatgggagacgctctcaccagctatgcaagccaccattgaaggtctaaacgtggttcactcagctactaaggtcttcggaagtctttaccaggcgacgaattggaggttcagtaacaccagtgtgaaggtgatggatgtggacgctggagacagggagacggtgcatccactcgtagttacacaccctgtaactggacgcagagccctttactgcaaccagatttactgccagaagatccagggaatgactgatgcggagtctaagtccctgcttcaattcctctacgaacacgccacccaattcgacttcacttgtcgtgttcggtggaagaaggaccaagtgctcgtgtgggataacctttgcaccatgcaccgagcagtaccagactacgccgggaaattccgctatctcacccgcactacagtggccggagacaagcctagccgctga

SEQ ID NO: 57 - DNA, 888 bp, Artificial Sequence
  Recombinant
atgcacgcggctttgacacctttgaccaacaagtatcggttcatcgacgttcaaccactcacaggcgtgctcggcgcagagattaccggagtggacctgagggagcccttagacgactccacttggaacgagatcctcgacgcctttcacacctaccaagttatctactttcctggacaggcgatcaccaacgagcagcacattgccttctcaaggaggttcggaccggtagatccagttccaattctcaaatccattgagggttatcccgaggtgcagatgattagacgagaagccaacgagtcctcacggtacataggcgacgattggcacgcagacagcaccttccttgacgctcctccggctgccgtggttatgcgcgcaatagaggtgccggagtacggcggcgataccggtttcctatcaatgtactctgcatgggagacgctctcaccaacgatgcaagccaccattgaaggtctaaacgtggttcactcagctactaaggtcttcggaagtctttaccaggcgacgaattggaggttcagtaacaccagtgtgaaggtgatggatgtggacgctggagacagggagacggtgcatccactcgtagttacacaccctgtaactggacgcagagccctttactgcaaccagatttactgccagaagatccagggaatgactgatgcggagtctaagtccctgcttcaattcctctacgaacacgccacccaattcgacttcacttgtcgtgttcggtggaagaaggaccaagtgctcgtgtgggataacctttgcaccatgcaccgagcagtaccagactacgccgggaaattccgctatctcacccgcactacagtggccggagacaagcctagccgctga

SEQ ID NO: 58 - DNA, 888 bp, Artificial Sequence
  Recombinant
atgcacgcggctttgacacctttgaccaacaagtatcggttcatcgacgttcaaccactcacaggcgtgctcggcgcagagattaccggagtggacctgagggagcccttagacgactccacttggaacgagatcctcgacgcctttcacacctaccaagttatctactttcctggacaggcgatcaccaacgagcagcacattgccttctcaaggaggttcggaccggtagatccagttccaattctcaaatccattgagggttatcccgaggtgcagatgattagacgagaagccaacgagtcctcacggtacataggcgacgattggcacgcagacagcaccttccttgacgctcctccggctgccgtggttatgcgcgcaatagaggtgccggagtacggcggcgataccggtttcctatcaatgtactctgcatgggagacgctctcaccaacgatgcaagccaccattgaaggtctaaacgtggttcactcagctactaaggtcttcggaagtctttaccaggcgacgaattggaggttcagtaacaccagtgtgaaggtgatggatgtggacgctggagacagggagacggtgcatccactcgtagttacacaccctgtaactggacgcagagccctttactgcaaccaggtttactgccagaagatccagggaatgactgatgcggagtctaagtccctgcttcaattcctctacgaacacgccacccaattcgacttcacttgtcgtgttcggtggaagaaggaccaagtgctcgtgtgggataacctttgcaccatgcaccgagcagtaccagactacgccgggaaattccgctatctcacccgcactacagtggccggagacaagcctagccgctga

SEQ ID NO: 59 - DNA, 888 bp, Artificial Sequence
  Recombinant
atgcacgcggctttgacacctttgaccaacaagtatcggcatatcgacgttcaaccactcacaggcgtgctcggcgcagagattaccggagtggacctgagggagcccttagacgactccacttggaacgagatcctcgacgcctttcacacctaccaagttatctactttcctggacaggcgatcaccaacgagcagcacattgccttctcaaggaggttcggaccggtagatccagttccaattctcaaatccattgagggttatcccgaggtgcagatgattagacgagaagccaacgagtcctcacggtacataggcgacgattggcacgcagacagcaccttccttgacgctcctccggctgccgtggttatgcgcgcaatagaggtgccggagtacggcggcgataccggtttcctatcaatgtactctgcatgggagacgctctcaccaacgatgcaagccaccattgaaggtctaaacgtggttcactcagctactaaggtcttcggaagtctttaccaggcgacgaattggaggttcagtaacaccagtgtgaaggtgatggatgtggacgctggagacagggagacggtgcatccactcgtagttacacaccctgtaactggacgcagagccctttactgcaaccaggtttactgccagaagatccagggaatgactgatgcggagtctaagtccctgcttcaattcctctacgaacacgccacccaattcgacttcacttgtcgtgttcggtggaagaaggaccaagtgctcgtgtgggataacctttgcaccatgcaccgagcagtaccagactacgccgggaaattccgctatctcacccgcactacagtggccggagacaagcctagccgctga

SEQ ID NO: 60 - protein, 295 aa, Sphingobium herbicidovorans
MHAALSPLSQRFERIAVQPLTGVLGAEITGVDLREPLDDSTWNEILDAFHTYQVIYFPGQAITNEQHIAFSRRFGPVDPVPLLKSIEGYPEVQMIRREANESGRVIGDDWHTDSTFLDAPPAAVVMRAIDVPEHGGDTGFLSMYTAWETLSPTMQATIEGLNVVHSATRVFGSLYQAQNRRFSNTSVKVMDVDAGDRETVHPLVVTHPGSGRKGLYVNQVYCQRIEGMTDAESKPLLQFLYEHATRFDFTCRVRWKKDQVLVWDNLCTMHRAVPDYAGKFRYLTRTTVGGVRPAR

SEQ ID NO: 61 - protein, 295 aa, Artificial Sequence
  consensus sequence
  misc_feature (6)..(6): Xaa can be any naturally occurring amino acid
  misc_feature (9)..(14): Xaa can be any naturally occurring amino acid
  misc_feature (16)..(16): Xaa can be any naturally occurring amino acid
  MISC_FEATURE (21)..(21): Thr can be Cys
  MISC_FEATURE (32)..(32): Asp can be Thr
  MISC_FEATURE (38)..(38): Asp can be Ser
  MISC_FEATURE (40)..(40): Ser can be Asn
  MISC_FEATURE (59)..(59): Gly can be Ala
  MISC_FEATURE (61)..(61): Ala can be Gln
  MISC_FEATURE (67)..(67): His can be Gln
  MISC_FEATURE (69)..(69): Ala can be Ser
  misc_feature (82)..(82): Xaa can be any naturally occurring amino acid
  misc_feature (103)..(103): Xaa can be any naturally occurring amino acid
  misc_feature (105)..(105): Xaa can be any naturally occurring amino acid
  MISC_FEATURE (106)..(106): Ile can be Leu
  MISC_FEATURE (108)..(108): Asp can be Glu
  MISC_FEATURE (109)..(109): Asp can be Asn
  misc_feature (112)..(112): Xaa can be any naturally occurring amino acid
  MISC_FEATURE (115)..(115): Thr can be Ser
  MISC_FEATURE (127)..(127): Arg can be Tyr
  MISC_FEATURE (129)..(129): Ile can be Arg or Lys
  MISC_FEATURE (130)..(130): Glu can be Asp
  MISC_FEATURE (131)..(131): Val can be Ile
  MISC_FEATURE (133)..(133): Glu can be Pro
  MISC_FEATURE (134)..(134): Tyr can be His
  MISC_FEATURE (139)..(139): Gly can be Leu
  MISC_FEATURE (141)..(141): Leu can be Thr or Ala
  misc_feature (145)..(145): Xaa can be any naturally occurring amino acid
  MISC_FEATURE (147)..(147): Trp can be Tyr
  misc_feature (148)..(148): Xaa can be any naturally occurring amino acid
  MISC_FEATURE (149)..(149): Thr can be Ala
  misc_feature (152)..(152): Xaa can be any naturally occurring amino acid
  MISC_FEATURE (153)..(153): Thr can be Gly or Ala
  MISC_FEATURE (154)..(154): Met can be Leu
  misc_feature (155)..(155): Xaa can be any naturally occurring amino acid
  MISC_FEATURE (156)..(156): Ala can be Lys
  MISC_FEATURE (157)..(157): Thr can be Leu
  MISC_FEATURE (159)..(159): Glu can be Ser
  misc_feature (169)..(169): Xaa can be any naturally occurring amino acid
  misc_feature (178)..(178): Xaa can be any naturally occurring amino acid
  misc_feature (180)..(180): Xaa can be any naturally occurring amino acid
  MISC_FEATURE (182)..(182): Phe can be Tyr
  MISC_FEATURE (184)..(184): Asn can be Gly
  MISC_FEATURE (193)..(193): Asp can be Ala
  MISC_FEATURE (194)..(194): Ala can be Asp
  MISC_FEATURE (206)..(206): Thr can be Ser
  misc_feature (209)..(209): Xaa can be any naturally occurring amino acid
  MISC_FEATURE (210)..(210): Thr can be Ser
  misc_feature (213)..(214): Xaa can be any naturally occurring amino acid
  misc_feature (217)..(217): Xaa can be any naturally occurring amino acid
  MISC_FEATURE (220)..(220): Val can be Ile
  misc_feature (224)..(224): Xaa can be any naturally occurring amino acid
  misc_feature (226)..(226): Xaa can be any naturally occurring amino acid
  MISC_FEATURE (229)..(229): Thr can be Ser
  MISC_FEATURE (230)..(230): Asp can be Glu
  MISC_FEATURE (231)..(231): Ala can be Lys
  MISC_FEATURE (234)..(234): Lys can be Glu
  misc_feature (235)..(235): Xaa can be any naturally occurring amino acid
  MISC_FEATURE (238)..(238): Gln can be Ser
  MISC_FEATURE (241)..(241): Tyr can be Phe
  MISC_FEATURE (242)..(242): Glu can be Ala
  misc_feature (246)..(246): Xaa can be any naturally occurring amino acid
  MISC_FEATURE (247)..(247): Phe can be Pro
  MISC_FEATURE (248)..(248): Asp can be Glu
  MISC_FEATURE (256)..(256): Lys can be Gln
  MISC_FEATURE (257)..(257): Lys can be Glu
  MISC_FEATURE (258)..(258): Asp can be Gly
  MISC_FEATURE (259)..(259): Gln can be Asp
  MISC_FEATURE (269)..(269): Met can be Gln
  misc_feature (271)..(271): Xaa can be any naturally occurring amino acid
  MISC_FEATURE (272)..(272): Ala can be Ser
  MISC_FEATURE (273)..(273): Val can be Ala or Ile
  MISC_FEATURE (274)..(274): Pro can be Asn
  MISC_FEATURE (277)..(277): Ala can be Asp or Gly or His
  MISC_FEATURE (278)..(278): Gly can be Asn
  MISC_FEATURE (279)..(279): Lys can be Ala or Gln
  MISC_FEATURE (280)..(280): Phe can be Thr
  MISC_FEATURE (282)..(282): Tyr can be Ile
  MISC_FEATURE (284)..(284): Thr can be His
  misc_feature (289)..(289): Xaa can be any naturally occurring amino acid
  misc_feature (291)..(292): Xaa can be any naturally occurring amino acid
  misc_feature (294)..(294): Xaa can be any naturally occurring amino acid
MHAALXPLXXXXXXIXVQPLTGVLGAEITGVDLREPLDDSTWNEILDAFHTYQVIYFPGQAITNEQHIAFSRRFGPVDPVPXLKSIEGYPEVQMIRREANESXRXIGDDWHXDSTFLDAPPAAVVMRAIEVPEYGGDTGFLSMYXAWXTLSXTMXATIEGLNVVHSATXVFGSLYQAXNXRFSNTSVKVMDVDAGDRETVHPLVVTHPXTGRXXLYXNQVYCQXIXGMTDAESKXLLQFLYEHATXFDFTCRVRWKKDQVLVWDNLCTMHXAVPDYAGKFRYLTRTTVXGXXPXR